European Patent Application EP 4 166 570 A1, published April 19, 2023. Title: RECOMBINANT FUSION PROTEINS TARGETING CD47 AND CD24, PREPARATION AND USE THEREOF. Applicant: ImmuneOnco Biopharmaceuticals (Shanghai) Co., Ltd. The sequence listing filed with the application follows.

SEQUENCE LISTING (36 sequences)

SEQ ID NO: 1 - protein, 125 aa, Artificial Sequence
  first extracellular Ig-like domain of SIRPalpha with mutation (SIRPalphaD1)
EEELQVIQPDKSVSVAAGESAILHCTVTSLIPVGPIQWFRGAGPARELIYNQKEGHFPRVTTVSESTKRENMDFSISISAITPADAGTYYCVKFRKGSPDTEFKSGAGTELSVRAKPSAPVVSGP

SEQ ID NO: 2 - protein, 117 aa, Artificial Sequence
  IMM47 and IMM47C's heavy chain variable region
DVQLQESGPDLVKPSQSLSLTCTVTGYSITSGYSWHWIRQFPGNKLEWMGYIHYSGSTKYNPSLKSRISITRDTSKNQFFLQLNSVTTEDTATYFCARGADYALDYWGQRTSVTVSS

SEQ ID NO: 3 - protein, 113 aa, Artificial Sequence
  IMM47's light chain variable region
DIQMTQSPSSLSASVGDRVTITCKSSQSLLYSSNQKNYLAWYQQKPGKAPKLLIYWASTRESGVPSRFSGSGSGTDFTLTISSLQPEDFATYYCQQNFIYPLTFGGGTKVELK

SEQ ID NO: 4 - protein, 113 aa, Artificial Sequence
  IMM47C's light chain variable region
DIVMSQSPSSLAVSVGEKVTMSCKSSQSLLYSSNQKNYLAWYQQKPGHSPKLLIYWASTRESGVPDRFTGSGSGTDFTLTISSVKAEDLAVYYCQQNFIYPLTFGAGTKLELK

SEQ ID NO: 5 - protein, 117 aa, Artificial Sequence
  IMM47H's heavy chain variable region
DVQLQESGPGLVKPSETLSLTCTVSGYSITSGYSWHWIRQPPGKGLEWIGYIHYSGSTKYNPSLKSRVTISVDTSKNQFSLKLSSVTAADTAVYYCARGADYALDYWGQRTSVTVSS

SEQ ID NO: 6 - protein, 113 aa, Artificial Sequence
  IMM47H's light chain variable region
DIVMTQSPDSLAVSLGERATINCKSSQSLLYSSNQKNYLAWYQQKPGQPPKLLIYWASTRESGVPDRFSGSGSGTDFTLTISSLQAEDVAVYYCQQNFIYPLTFGGGTKVELK

SEQ ID NO: 7 - protein, 9 aa, Artificial Sequence
  IMM47, IMM47C and IMM47H's heavy chain CDR1 (HV-CDR-1)
GYSITSGYS

SEQ ID NO: 8 - protein, 7 aa, Artificial Sequence
  IMM47, IMM47C and IMM47H's heavy chain CDR2 (HV-CDR-2)
IHYSGST

SEQ ID NO: 9 - protein, 10 aa, Artificial Sequence
  IMM47, IMM47C and IMM47H's heavy chain CDR3 (HV-CDR-3)
ARGADYALDY

SEQ ID NO: 10 - protein, 12 aa, Artificial Sequence
  IMM47, IMM47C and IMM47H's light chain CDR1 (LV-CDR-1)
QSLLYSSNQKNY

SEQ ID NO: 11 - protein, 3 aa, Artificial Sequence
  IMM47, IMM47C and IMM47H's light chain CDR2 (LV-CDR-2)
WAS

SEQ ID NO: 12 - protein, 9 aa, Artificial Sequence
  IMM47, IMM47C and IMM47H's light chain CDR3 (LV-CDR-3)
QQNFIYPLT

SEQ ID NO: 13 - protein, 330 aa, Artificial Sequence
  IMM47, IMM47C and IMM47H's heavy chain constant region
ASTKGPSVFPLAPSSKSTSGGTAALGCLVKDYFPEPVTVSWNSGALTSGVHTFPAVLQSSGLYSLSSVVTVPSSSLGTQTYICNVNHKPSNTKVDKRVEPKSCDKTHTCPPCPAPELLGGPSVFLFPPKPKDTLMISRTPEVTCVVVDVSHEDPEVKFNWYVDGVEVHNAKTKPREEQYNATYRVVSVLTVLHQDWLNGKEYKCKVSNKALPAPIAATISKAKGQPREPQVYTLPPSREEMTKNQVSLTCLVKGFYPSDIAVEWESNGQPENNYKTTPPVLDSDGSFFLYSKLTVDKSRWQQGNVFSCSVMHEALHNHYTQKSLSLSPGK

SEQ ID NO: 14 - protein, 107 aa, Artificial Sequence [sequence omitted]

SEQ ID NO: 15 - protein, 15 aa, Artificial Sequence
  Linker
GGGGSGGGGSGGGGS

SEQ ID NO: 16 - protein, 10 aa, Artificial Sequence
  Linker
GGGGSGGGGS

SEQ ID NO: 17 - protein, 20 aa, Artificial Sequence
  Linker
GGGGSGGGGSGGGGSGGGGS

SEQ ID NO: 18 - protein, 587 aa, Artificial Sequence
  IMM4701C's long chain (SIRPalphaD1-linker-IMM47C's heavy chain)
EEELQVIQPDKSVSVAAGESAILHCTVTSLIPVGPIQWFRGAGPARELIYNQKEGHFPRVTTVSESTKRENMDFSISISAITPADAGTYYCVKFRKGSPDTEFKSGAGTELSVRAKPSAPVVSGPGGGGSGGGGSGGGGSDVQLQESGPDLVKPSQSLSLTCTVTGYSITSGYSWHWIRQFPGNKLEWMGYIHYSGSTKYNPSLKSRISITRDTSKNQFFLQLNSVTTEDTATYFCARGADYALDYWGQRTSVTVSSASTKGPSVFPLAPSSKSTSGGTAALGCLVKDYFPEPVTVSWNSGALTSGVHTFPAVLQSSGLYSLSSVVTVPSSSLGTQTYICNVNHKPSNTKVDKRVEPKSCDKTHTCPPCPAPELLGGPSVFLFPPKPKDTLMISRTPEVTCVVVDVSHEDPEVKFNWYVDGVEVHNAKTKPREEQYNATYRVVSVLTVLHQDWLNGKEYKCKVSNKALPAPIAATISKAKGQPREPQVYTLPPSREEMTKNQVSLTCLVKGFYPSDIAVEWESNGQPENNYKTTPPVLDSDGSFFLYSKLTVDKSRWQQGNVFSCSVMHEALHNHYTQKSLSLSPGK

SEQ ID NO: 19 - DNA, 1821 bp, Artificial Sequence
  IMM4701C's long chain (SIRPalphaD1-linker-IMM47C's heavy chain)
atgggatggtcatgtatcatcctttttctggtagcaactgcaactggagtacattcagaggaggagctgcaggtgattcagcctgacaagtccgtatcagttgcagctggagagtcggccattctgcactgcactgtgacctccctgatccctgtggggcccatccagtggttcagaggagctggaccagcccgggaattaatctacaatcaaaaagaaggccacttcccccgggtaacaactgtttcagagtccacaaagagagaaaacatggacttttccatcagcatcagtgccatcaccccagcagatgccggcacctactactgtgtgaagttccggaaagggagccctgacacggagtttaagtctggagcaggcactgagctgtctgtgcgtgccaaaccctctgcccccgtggtatcgggccctggcggcggtgggagcggcggcggtgggagcggcggcgggggctcggatgtgcagcttcaggagtcaggacctgacctggtgaaaccttctcagtcactttcactcacctgcactgtcactggctactccatcaccagtggttatagctggcactggatccggcagtttccaggaaacaaactggaatggatgggctacatacactatagtggtagcactaagtacaacccatctctcaaaagtcgaatctctatcactcgagacacatccaagaaccagttcttcctgcagttgaattctgtgactactgaggacacagccacatatttctgtgcaagaggcgcggactatgctttggactactggggtcaacgaacctcagtcaccgtctcctcagctagcaccaagggcccatcggtcttccccctggcaccctcctccaagagcacctctgggggcacagcggccctgggctgcctggtcaaggactacttccccgaaccggtgacggtgtcgtggaactcaggcgccctgaccagcggcgtgcacaccttcccggctgtcctacagtcctcaggactctactccctcagcagcgtggtgaccgtgccctccagcagcttgggcacccagacctacatctgcaacgtgaatcacaagcccagcaacaccaaggtggacaagagagttgagcccaaatcttgtgacaaaactcacacatgcccaccgtgcccagcacctgaactcctggggggaccgtcagtcttcctcttccccccaaaacccaaggacaccctcatgatctcccggacccctgaggtcacatgcgtggtggtggacgtgagccacgaagaccctgaggtcaagttcaactggtatgtggacggcgtggaggtgcataatgccaagacaaagccgcgggaggagcagtacaacgccacgtaccgtgtggtcagcgtcctcaccgtcctgcaccaagactggctgaatggcaaggagtacaagtgcaaggtctccaacaaagccctcccagcccccatcgccgcaaccatctccaaagccaaagggcagccccgagaaccacaggtgtacaccctgcccccatcccgggaggagatgaccaagaaccaagtcagcctgacctgcctggtcaaaggcttctatcccagcgacatcgccgtggagtgggagagcaatgggcagccggagaacaactacaagaccacgcctcccgtgctggactccgacggctccttcttcctctattccaagctcaccgtggacaagagcaggtggcagcaggggaacgtcttctcatgctccgtgatgcatgaggctctgcacaaccactacacgcagaagagcctctccctgtctccgggcaaatga

SEQ ID NO: 20 - protein, 220 aa, Artificial Sequence
  IMM4701C's short chain (IMM47C's light chain)
DIVMSQSPSSLAVSVGEKVTMSCKSSQSLLYSSNQKNYLAWYQQKPGHSPKLLIYWASTRESGVPDRFTGSGSGTDFTLTISSVKAEDLAVYYCQQNFIYPLTFGAGTKLELKRTVAAPSVFIFPPSDEQLKSGTASVVCLLNNFYPREAKVQWKVDNALQSGNSQESVTEQDSKDSTYSLSSTLTLSKADYEKHKVYACEVTHQGLSSPVTKSFNRGEC

SEQ ID NO: 21 - DNA, 862 bp, Artificial Sequence
  IMM4701C's short chain (IMM47C's light chain)
atggattcacaggcccaggttcttatgttactgctgctatgggtatctggtacctgtggggacattgtgatgtcacagtctccatcctccctagctgtgtcagttggagagaaggttactatgagctgcaagtccagtcagagccttttatatagtagcaatcaaaagaactacttggcctggtaccagcagaaaccagggcactctcctaaactgctgatttactgggcatccactagggaatctggggtccctgatcgcttcacaggcagtggatctgggacagatttcactctcaccatcagcagtgtgaaggctgaagacctggcagtttattactgtcagcaaaattttatctatccgctcacgttcggtgctgggaccaagctggagctgaaacgtgagttctagaggatccatctgggataagcatgctgttttctgtctgtccctaacatgccctgtgattatccgcaaacaacacacccaagggcagaactttgttacttaaacaccatcctgtttgcttctttcctcaggaactgtggctgcaccatctgtcttcatcttcccgccatctgatgagcagttgaaatctggaactgcctctgttgtgtgcctgctgaataacttctatcccagagaggccaaagtacagtggaaggtggataacgccctccaatcgggtaactcccaggagagtgtcacagagcaggacagcaaggacagcacctacagcctcagcagcaccctgacgctgagcaaagcagactacgagaaacacaaagtctacgcctgcgaagtcacccatcagggcctgagctcgcccgtcacaaagagcttcaacaggggagagtgttag

SEQ ID NO: 22 - protein, 220 aa, Artificial Sequence
  IMM4701's short chain (IMM47's light chain)
DIQMTQSPSSLSASVGDRVTITCKSSQSLLYSSNQKNYLAWYQQKPGKAPKLLIYWASTRESGVPSRFSGSGSGTDFTLTISSLQPEDFATYYCQQNFIYPLTFGGGTKVELKRTVAAPSVFIFPPSDEQLKSGTASVVCLLNNFYPREAKVQWKVDNALQSGNSQESVTEQDSKDSTYSLSSTLTLSKADYEKHKVYACEVTHQGLSSPVTKSFNRGEC

SEQ ID NO: 23 - DNA, 859 bp, Artificial Sequence
  IMM4701's short chain (IMM47's light chain)
atgggatggtcatgtatcatcctttttctggtagcaactgcaactggagtacattcagacattcagatgacacagagccctagcagcctgagcgcctccgtgggcgacagagtgaccatcacctgcaagagcagccaaagcctgctgtacagcagcaatcagaagaactacctggcctggtatcagcagaagcctggcaaggcccctaagctgctgatctactgggcctccacaagagagagcggcgtgcctagcagattcagcggcagcggcagcggcaccgacttcaccctgaccatcagcagcctgcagcctgaggacttcgccacctactactgtcagcagaacttcatctaccctctgaccttcggcggaggcaccaaggtggagctgaagcgtgagttctagaggatccatctgggataagcatgctgttttctgtctgtccctaacatgccctgtgattatccgcaaacaacacacccaagggcagaactttgttacttaaacaccatcctgtttgcttctttcctcaggaactgtggctgcaccatctgtcttcatcttcccgccatctgatgagcagttgaaatctggaactgcctctgttgtgtgcctgctgaataacttctatcccagagaggccaaagtacagtggaaggtggataacgccctccaatcgggtaactcccaggagagtgtcacagagcaggacagcaaggacagcacctacagcctcagcagcaccctgacgctgagcaaagcagactacgagaaacacaaagtctacgcctgcgaagtcacccatcagggcctgagctcgcccgtcacaaagagcttcaacaggggagagtgttag

SEQ ID NO: 24 - protein, 447 aa, Artificial Sequence
  IMM4702C's long chain (IMM47C's heavy chain)
DVQLQESGPDLVKPSQSLSLTCTVTGYSITSGYSWHWIRQFPGNKLEWMGYIHYSGSTKYNPSLKSRISITRDTSKNQFFLQLNSVTTEDTATYFCARGADYALDYWGQRTSVTVSSASTKGPSVFPLAPSSKSTSGGTAALGCLVKDYFPEPVTVSWNSGALTSGVHTFPAVLQSSGLYSLSSVVTVPSSSLGTQTYICNVNHKPSNTKVDKRVEPKSCDKTHTCPPCPAPELLGGPSVFLFPPKPKDTLMISRTPEVTCVVVDVSHEDPEVKFNWYVDGVEVHNAKTKPREEQYNATYRVVSVLTVLHQDWLNGKEYKCKVSNKALPAPIAATISKAKGQPREPQVYTLPPSREEMTKNQVSLTCLVKGFYPSDIAVEWESNGQPENNYKTTPPVLDSDGSFFLYSKLTVDKSRWQQGNVFSCSVMHEALHNHYTQKSLSLSPGK

SEQ ID NO: 25 - DNA, 1398 bp, Artificial Sequence
  IMM4702C's long chain (IMM47C's heavy chain)
atgagagtgctgattcttttgtgcctgttcacagcctttcctggtatcctgtctgatgtgcagcttcaggagtcaggacctgacctggtgaaaccttctcagtcactttcactcacctgcactgtcactggctactccatcaccagtggttatagctggcactggatccggcagtttccaggaaacaaactggaatggatgggctacatacactatagtggtagcactaagtacaacccatctctcaaaagtcgaatctctatcactcgagacacatccaagaaccagttcttcctgcagttgaattctgtgactactgaggacacagccacatatttctgtgcaagaggcgcggactatgctttggactactggggtcaacgaacctcagtcaccgtctcctcagctagcaccaagggcccatcggtcttccccctggcaccctcctccaagagcacctctgggggcacagcggccctgggctgcctggtcaaggactacttccccgaaccggtgacggtgtcgtggaactcaggcgccctgaccagcggcgtgcacaccttcccggctgtcctacagtcctcaggactctactccctcagcagcgtggtgaccgtgccctccagcagcttgggcacccagacctacatctgcaacgtgaatcacaagcccagcaacaccaaggtggacaagagagttgagcccaaatcttgtgacaaaactcacacatgcccaccgtgcccagcacctgaactcctggggggaccgtcagtcttcctcttccccccaaaacccaaggacaccctcatgatctcccggacccctgaggtcacatgcgtggtggtggacgtgagccacgaagaccctgaggtcaagttcaactggtatgtggacggcgtggaggtgcataatgccaagacaaagccgcgggaggagcagtacaacgccacgtaccgtgtggtcagcgtcctcaccgtcctgcaccaagactggctgaatggcaaggagtacaagtgcaaggtctccaacaaagccctcccagcccccatcgccgcaaccatctccaaagccaaagggcagccccgagaaccacaggtgtacaccctgcccccatcccgggaggagatgaccaagaaccaagtcagcctgacctgcctggtcaaaggcttctatcccagcgacatcgccgtggagtgggagagcaatgggcagccggagaacaactacaagaccacgcctcccgtgctggactccgacggctccttcttcctctattccaagctcaccgtggacaagagcaggtggcagcaggggaacgtcttctcatgctccgtgatgcatgaggctctgcacaaccactacacgcagaagagcctctccctgtctccgggcaaatga

SEQ ID NO: 26 - protein, 360 aa, Artificial Sequence
  IMM4702C's short chain (SIRPalphaD1-linker-IMM47C's light chain)
EEELQVIQPDKSVSVAAGESAILHCTVTSLIPVGPIQWFRGAGPARELIYNQKEGHFPRVTTVSESTKRENMDFSISISAITPADAGTYYCVKFRKGSPDTEFKSGAGTELSVRAKPSAPVVSGPGGGGSGGGGSGGGGSDIVMSQSPSSLAVSVGEKVTMSCKSSQSLLYSSNQKNYLAWYQQKPGHSPKLLIYWASTRESGVPDRFTGSGSGTDFTLTISSVKAEDLAVYYCQQNFIYPLTFGAGTKLELKRTVAAPSVFIFPPSDEQLKSGTASVVCLLNNFYPREAKVQWKVDNALQSGNSQESVTEQDSKDSTYSLSSTLTLSKADYEKHKVYACEVTHQGLSSPVTKSFNRGEC

SEQ ID NO: 27 - DNA, 1279 bp, Artificial Sequence
  IMM4702C's short chain (SIRPalphaD1-linker-IMM47C's light chain)
atgggatggtcatgtatcatcctttttctggtagcaactgcaactggagtacattcagaggaggagctgcaggtgattcagcctgacaagtccgtatcagttgcagctggagagtcggccattctgcactgcactgtgacctccctgatccctgtggggcccatccagtggttcagaggagctggaccagcccgggaattaatctacaatcaaaaagaaggccacttcccccgggtaacaactgtttcagagtccacaaagagagaaaacatggacttttccatcagcatcagtgccatcaccccagcagatgccggcacctactactgtgtgaagttccggaaagggagccctgacacggagtttaagtctggagcaggcactgagctgtctgtgcgtgccaaaccctctgcccccgtggtatcgggccctggcggcggtgggagcggcggcggtgggagcggcggcgggggctcggacattgtgatgtcacagtctccatcctccctagctgtgtcagttggagagaaggttactatgagctgcaagtccagtcagagccttttatatagtagcaatcaaaagaactacttggcctggtaccagcagaaaccagggcactctcctaaactgctgatttactgggcatccactagggaatctggggtccctgatcgcttcacaggcagtggatctgggacagatttcactctcaccatcagcagtgtgaaggctgaagacctggcagtttattactgtcagcaaaattttatctatccgctcacgttcggtgctgggaccaagctggagctgaagcgtgagttctagaggatccatctgggataagcatgctgttttctgtctgtccctaacatgccctgtgattatccgcaaacaacacacccaagggcagaactttgttacttaaacaccatcctgtttgcttctttcctcaggaactgtggctgcaccatctgtcttcatcttcccgccatctgatgagcagttgaaatctggaactgcctctgttgtgtgcctgctgaataacttctatcccagagaggccaaagtacagtggaaggtggataacgccctccaatcgggtaactcccaggagagtgtcacagagcaggacagcaaggacagcacctacagcctcagcagcaccctgacgctgagcaaagcagactacgagaaacacaaagtctacgcctgcgaagtcacccatcagggcctgagctcgcccgtcacaaagagcttcaacaggggagagtgttag

SEQ ID NO: 28 - protein, 447 aa, Artificial Sequence
  IMM4702H's long chain (IMM47H's heavy chain)
DVQLQESGPGLVKPSETLSLTCTVSGYSITSGYSWHWIRQPPGKGLEWIGYIHYSGSTKYNPSLKSRVTISVDTSKNQFSLKLSSVTAADTAVYYCARGADYALDYWGQRTSVTVSSASTKGPSVFPLAPSSKSTSGGTAALGCLVKDYFPEPVTVSWNSGALTSGVHTFPAVLQSSGLYSLSSVVTVPSSSLGTQTYICNVNHKPSNTKVDKRVEPKSCDKTHTCPPCPAPELLGGPSVFLFPPKPKDTLMISRTPEVTCVVVDVSHEDPEVKFNWYVDGVEVHNAKTKPREEQYNATYRVVSVLTVLHQDWLNGKEYKCKVSNKALPAPIAATISKAKGQPREPQVYTLPPSREEMTKNQVSLTCLVKGFYPSDIAVEWESNGQPENNYKTTPPVLDSDGSFFLYSKLTVDKSRWQQGNVFSCSVMHEALHNHYTQKSLSLSPGK

SEQ ID NO: 29 - DNA, 1401 bp, Artificial Sequence
  IMM4702H's long chain (IMM47H's heavy chain)
atgggatggtcatgtatcatcctttttctggtagcaactgcaactggagtacattcagacgtgcagctgcaagagagcggccctggcctggtgaagcctagcgagaccctgagcctgacctgcaccgtgtccggctacagcatcacaagcggctacagctggcactggatcagacagcctcctggcaagggcctggagtggatcggctacatccactacagcggcagcaccaagtacaaccctagcctgaagagcagagtgaccatcagcgtggacacaagcaagaatcagttcagcctgaagctgagcagcgtgaccgccgccgacaccgccgtgtactactgcgctagaggcgccgactacgccctggactactggggacagagaacaagcgtgaccgtgagcagcgctagcaccaagggcccatcggtcttccccctggcaccctcctccaagagcacctctgggggcacagcggccctgggctgcctggtcaaggactacttccccgaaccggtgacggtgtcgtggaactcaggcgccctgaccagcggcgtgcacaccttcccggctgtcctacagtcctcaggactctactccctcagcagcgtggtgaccgtgccctccagcagcttgggcacccagacctacatctgcaacgtgaatcacaagcccagcaacaccaaggtggacaagagagttgagcccaaatcttgtgacaaaactcacacatgcccaccgtgcccagcacctgaactcctggggggaccgtcagtcttcctcttccccccaaaacccaaggacaccctcatgatctcccggacccctgaggtcacatgcgtggtggtggacgtgagccacgaagaccctgaggtcaagttcaactggtatgtggacggcgtggaggtgcataatgccaagacaaagccgcgggaggagcagtacaacgccacgtaccgtgtggtcagcgtcctcaccgtcctgcaccaagactggctgaatggcaaggagtacaagtgcaaggtctccaacaaagccctcccagcccccatcgccgcaaccatctccaaagccaaagggcagccccgagaaccacaggtgtacaccctgcccccatcccgggaggagatgaccaagaaccaagtcagcctgacctgcctggtcaaaggcttctatcccagcgacatcgccgtggagtgggagagcaatgggcagccggagaacaactacaagaccacgcctcccgtgctggactccgacggctccttcttcctctattccaagctcaccgtggacaagagcaggtggcagcaggggaacgtcttctcatgctccgtgatgcatgaggctctgcacaaccactacacgcagaagagcctctccctgtctccgggcaaatga

SEQ ID NO: 30 - protein, 360 aa, Artificial Sequence
  IMM4702H's short chain (SIRPalphaD1-linker-IMM47H's light chain)
EEELQVIQPDKSVSVAAGESAILHCTVTSLIPVGPIQWFRGAGPARELIYNQKEGHFPRVTTVSESTKRENMDFSISISAITPADAGTYYCVKFRKGSPDTEFKSGAGTELSVRAKPSAPVVSGPGGGGSGGGGSGGGGSDIVMTQSPDSLAVSLGERATINCKSSQSLLYSSNQKNYLAWYQQKPGQPPKLLIYWASTRESGVPDRFSGSGSGTDFTLTISSLQAEDVAVYYCQQNFIYPLTFGGGTKVELKRTVAAPSVFIFPPSDEQLKSGTASVVCLLNNFYPREAKVQWKVDNALQSGNSQESVTEQDSKDSTYSLSSTLTLSKADYEKHKVYACEVTHQGLSSPVTKSFNRGEC

SEQ ID NO: 31 - DNA, 1279 bp, Artificial Sequence
  IMM4702H's short chain (SIRPalphaD1-linker-IMM47H's light chain)
atgggatggtcatgtatcatcctttttctggtagcaactgcaactggagtacattcagaggaggagctgcaggtgattcagcctgacaagtccgtatcagttgcagctggagagtcggccattctgcactgcactgtgacctccctgatccctgtggggcccatccagtggttcagaggagctggaccagcccgggaattaatctacaatcaaaaagaaggccacttcccccgggtaacaactgtttcagagtccacaaagagagaaaacatggacttttccatcagcatcagtgccatcaccccagcagatgccggcacctactactgtgtgaagttccggaaagggagccctgacacggagtttaagtctggagcaggcactgagctgtctgtgcgtgccaaaccctctgcccccgtggtatcgggccctggcggcggtgggagcggcggcggtgggagcggcggcgggggctcggacatcgtgatgacacagagccctgacagcctggccgtgagcctgggcgagagagccaccatcaactgcaagagctctcagagcctgctgtacagcagcaatcagaagaactacctggcctggtatcagcagaagcctggacagcctcctaagctgctgatctactgggcaagcacaagagagagcggcgtgcctgacagattcagcggcagcggcagcggcaccgacttcaccctgaccatcagcagcctgcaagccgaggacgtggccgtgtactactgtcagcagaacttcatctaccctctgaccttcggcggcggcaccaaggtggagctgaagcgtgagttctagaggatccatctgggataagcatgctgttttctgtctgtccctaacatgccctgtgattatccgcaaacaacacacccaagggcagaactttgttacttaaacaccatcctgtttgcttctttcctcaggaactgtggctgcaccatctgtcttcatcttcccgccatctgatgagcagttgaaatctggaactgcctctgttgtgtgcctgctgaataacttctatcccagagaggccaaagtacagtggaaggtggataacgccctccaatcgggtaactcccaggagagtgtcacagagcaggacagcaaggacagcacctacagcctcagcagcaccctgacgctgagcaaagcagactacgagaaacacaaagtctacgcctgcgaagtcacccatcagggcctgagctcgcccgtcacaaagagcttcaacaggggagagtgttag

SEQ ID NO: 32 - protein, 364 aa, Artificial Sequence
  SIRPalphaD1 mutant-Fc (IMM01)
EEELQVIQPDKSVSVAAGESAILHCTVTSLIPVGPIQWFRGAGPARELIYNQKEGHFPRVTTVSESTKRENMDFSISISAITPADAGTYYCVKFRKGSPDTEFKSGAGTELSVRAKPSAPVVSGPAARATPQHEPKSCDKTHTCPPCPAPELLGGPSVFLFPPKPKDTLMISRTPEVTCVVVDVSHEDPEVKFNWYVDGVEVHNAKTKPREEQYNSTYRVVSVLTVLHQDWLNGKEYKCKVSNKALPAPIEKTISKAKGQPREPQVYTLPPSRDELTKNQVSLTCLVKGFYPSDIAVEWESNGQPENNYKTTPPVLDSDGSFFLYSKLTVDKSRWQQGNVFSCSVMHEALHNHYTQKSLSLSPG

SEQ ID NO: 33 - DNA, 1095 bp, Artificial Sequence
  SIRPalphaD1 mutant-Fc (IMM01)
gaggaggagctgcaggtgattcagcctgacaagtccgtatcagttgcagctggagagtcggccattctgcactgcactgtgacctccctgatccctgtggggcccatccagtggttcagaggagctggaccagcccgggaattaatctacaatcaaaaagaaggccacttcccccgggtaacaactgtttcagagtccacaaagagagaaaacatggacttttccatcagcatcagtgccatcaccccagcagatgccggcacctactactgtgtgaagttccggaaagggagccctgacacggagtttaagtctggagcaggcactgagctgtctgtgcgtgccaaaccctctgcccccgtggtatcgggccctgcggcgagggccacacctcagcacgagcccaaatcttgtgacaaaactcacacatgcccaccgtgcccagcacctgaactcctggggggaccgtcagtcttcctcttccccccaaaacccaaggacaccctcatgatctcccggacccctgaggtcacatgcgtggtggtggacgtgagccacgaagaccctgaggtcaagttcaactggtacgtggacggcgtggaggtgcataatgccaagacaaagccgcgggaggagcagtacaacagcacgtaccgtgtggtcagcgtcctcaccgtcctgcaccaggactggctgaatggcaaggagtacaagtgcaaggtctccaacaaagccctcccagcccccatcgagaaaaccatctccaaagccaaagggcagccccgagaaccacaggtgtacaccctgcccccatcccgggatgagctgaccaagaaccaggtcagcctgacctgcctggtcaaaggcttctatcccagcgacatcgccgtggagtgggagagcaatgggcagccggagaacaactacaagaccacgcctcccgtgctggactccgacggctccttcttcctctacagcaagctcaccgtggacaagagcaggtggcagcaggggaacgtcttctcatgctccgtgatgcatgaggctctgcacaaccactacacgcagaagagcctctccctgtctccgggttga

SEQ ID NO: 34 - DNA, 57 bp, Artificial Sequence
  nucleotide encoding mouse IgG1 heavy chain signal peptide
atgggatggtcatgtatcatcctttttctggtagcaactgcaactggagtacattca

SEQ ID NO: 35 - DNA, 9 bp, Artificial Sequence
  Kozak consensus sequence
gccgccacc

SEQ ID NO: 36 - protein, 597 aa, Artificial Sequence
  human SIRPalpha-mouse IgG1 Fc
MGWSCIILFLVATATGVHSSCAWSGVAGEEELQVIQPDKSVSVAAGESAILHCTVTSLIPVGPIQWFRGAGPARELIYNQKEGHFPRVTTVSESTKRENMDFSISISNITPADAGTYYCVKFRKGSPDTEFKSGAGTELSVRAKPSAPVVSGPAARATPQHTVSFTCESHGFSPRDITLKWFKNGNELSDFQTNVDPVGESVSYSIHSTAKVVLTREDVHSQVICEVAHVTLQGDPLRGTANLSETIRVPPTLEVTQQPVRAENQVNVTCQVRKFYPQRLQLTWLENGNVSRTETASTVTENKDGTYNWMSWLLVNVSAHRDDVKLTCQVEHDGQPAVSKSHDLKVSAHPKEQGSNTAAENTGSNERNEFVPRDCGCKPCICTVPEVSSVFIFPPKPKDVLTITLTPKVTCVVVDISKDDPEVQFSWFVDDVEVHTAQTQPREEQFNSTFRSVSELPIMHQDWLNGKEFKCRVNSAAFPAPIEKTISKTKGRPKAPQVYTIPPPKEQMAKDKVSLTCMITDFFPEDITVEWQWNGQPAENYKNTQPIMNTNGSYFVYSKLNVQKSNWEAGNTFTCSVLHEGLHNHHTEKSLSHSPGK